European Patent Specification EP 3 878 952 B1, published September 6, 2023. Title: FUNCTIONALIZATION OF ENDOGENOUS BACTERIA. Applicant: Massachusetts Institute of Technology Trustees of Boston University. Application Not Yet Assigned. The sequence listing filed with the application follows.

SEQUENCE LISTING (9 sequences)

SEQ ID NO: 1 - DNA, 6249 bp, Artificial Sequence
  Synthetic Polynucleotide
gacgtctgtgcaagtactactgttctgcagtcacttgaattcaagaaaccaatagtccatattgcatcagacattgccgtcactgcgtcttttactggctcttctcgctaaccaaaccggtaaccccgcttattaaaagcattctgtaacaaagcgggaccaaagccatgacaaaagcgcgtaacaaaagtgtctataatcacggcagaaaagtccacattgattatttgcacggcgtcacactttgctatgccatagcatttttatccataagattagcggatcatacctgacgctttttatcgcaactctctactgtttctccatacagctgaaaagcttacgggaggaacgttatgaatcagaccgacacatcacctatcaggctgcgcaggagctggaacaccagcgagatagaagcgctctttgacgagcatgccggacgtatcgatccgcgcatttataccgatgaggatctgtaccaactcgaactggagcgtgtcttcgcccggtcctggctgctgttggggcatgaaacccagattcgcaagccgggcgattacatcacgacctacatgggtgaagaccctgtcgtggtcgtccggcagaaagacgccagcattgccgtgttcctgaaccagtgccgccaccgtggcatgcgcatctgccgcgcggatgccggaaacgcgaaggcgttcacttgcagctaccacgggtgggcttacgacaccgccggcaatcttgtcaatgtgccttacgaggccgaatccttcgcgtgcctgaacaagaaggaatggagcccgctgaaggcccgggtagaaacctacaagggcctgattttcgccaactgggatgagaacgctgtagacctcgacacgtatctgggcgaggcgaagttctacatggaccacatgctcgaccgcaccgaggccggcaccgaagcgatcccgggcgtgcagaagtgggtcattccctgtaactggaaattcgccgcagagcagttttgcagcgacatgtaccatgccgggacgacctcgcatctgtctggcatcctggcaggcctgccagaagaccttgaaatggccgaccttgctccgccgacagttggcaagcagtaccgtgcgtcatggggcggacatggaagtggcttctatgtcggcgaccccaatctgatgcttgccatcatggggccaaaggtcaccagctactggaccgaaggccccgcgtcggaaaaggcggccgaacgtctgggtagcgtggagcgcggctcgaaactcatggtcgagcacatgaccgtcttccccacgtgttccttcctcccaggtatcaatacggtccggacatggcatccgcgcgggccgaacgaggtcgaggtatgggcgtttacggtggtcgatgctgatgctcctgacgatatcaaggaagagttccggcgccagacgctgcgcaccttctctgccggtggcgtgttcgagcaggacgacggggagaactgggtcgagatccagcacatcctgcgaggccacaaggcgcggagccgccctttcaatgccgagatgagcatggaccagaccgtcgacaacgacccggtttaccccgggcggatcagcaacaacgtctacagcgaggaagctgcccgcgggctctatgcccattggctgcggatgatgacatcccccgactgggacgcgctgaaggcgacacgctgaatccagagacagcttgcgccacgcagtggcgccggccagaggccgcatttgacttcgacccaggttggatgcggtggaccttgtccatttgaaatctacaaggaacgaccatgattgattcagccaacagagccgacgtctttctccgcaagccggcacccgtagcgcccgaactgcagcacgaagtcgagcagttctactattgggaggccaagcttctcaacgatcgccgcttcgaggagtggttcgcgctgctcgcggaagacattcactacttcatgcccattcgcaccacgcggatcatgcgggactcgcgccttgaatactcaggctcccgagagtacgcgcacttcgatgacgacgccacgatgatgaagggacgcttgcgcaagatcacgtccgacgtgagctggtccgagaaccccgcatcgcggacccggcatctcgtgagcaacgtgatgatcgtcggcgcagaggcagaaggggagtacgaaatctcaagcgccttcattgtgtaccgcaatcgtctggagcggcagctcgacatctttgccggtgagcgtcgcgatacgttgcgccgtaacacgagcgaggccgggttcgagatcgtcaatcggaccatcctgatcgaccagagcaccatcctggccaataacctcagtttcttcttctaggtgatgtcatgacttggacatacatattgcggcagggtgacctgccacccggtgagatgcagcgctacgaaggcggcccggaacctgtgatggtctgcaacgtcgatggcgagttcttcgcggtgcaggatacctgcacgcatggggactgggcgttgtcggatggttacctggacggtgatattgtcgaatgcacgttgcatttcggcaagttctgcgtgcggaccgggaaggtgaaggcgctgcctgcttgcaaacctatcaaggtattcccaatcaaggtcgaaggcgatgaagtgcacgtcgatctcgacaacggggagttgaagtgatggctacccatgtggcgatcatcggcaatggcgtgggtggcttcacgaccgcgcaggccctacgtgccgagggcttcgaggggagaatctcgctgattggggacgaaccgcatctcccctatgaccgaccatccttgtccaaggcggttctcgacggcagccttgagcggccgcccatactggccgaggccgattggtacggcgaggcccgcatcgacatgctgaccggcccggaagtcactgcccttgatgtgcagacaaggacgatcagtctggatgatggcaccacgctctctgcggacgccatcgtcatcgcgacgggcagtcgagcgcggacgatggcgttgcccggcagccaactgccgggcgtcgtaacgctgcgcacctacggtgacgtgcaggtattgcgcgatagttggacttccgcgacgcggctgctgattgtgggtggcggattgatcggctgcgaggtcgcgacgacggcgcgcaagctcggcctgtcggtcacgatcctggaggcaggtgatgaactgctggtccgagtacttgggcggcgtatcggtgcctggctgcgcggcctgctgacagaacttggtgtgcaggtcgagttgggaacgggtgtcgtaggtttttctggtgagggccagctcgaacaagtcatggccagcgatgggcgcagcttcgtagccgatagcgcactcatttgcgtcggcgcggagcccgcggatcaacttgcgcgtcaagcgggcttggcatgtgaccgcggcgtcattgtcgatcactgcggtgcgacgcttgccaaaggcgtattcgccgtcggagatgtggccagttggccgctgcgcgccggcggccggcgttcgctcgaaacctatatgaacgcgcagcgccaagccgccgcggtggctgcggccattctggggaaaaacgtatcggcaccgcaactgcccgtgtcctggacggagatcgctgggcatcgcatgcagatggcgggcgatatcgaaggacctggtgatttcgtctcgcgcggcatgcccggtagtggcgctgccctgttgttccgcctgcaggagcgaaggattcaggcggtcgtcgcggtcgatgcaccccgtgacttcgcgcttgcaacccgattggtagaagcccgcgcggcaatcgagccagcacggctggcagatctttcaaacagtatgcgcgattttgttcgtgcgaatgaaggagacctaacgtgaggtacccgagaattggcttggactcctgttgatagatccagtaatgacctcagaactccatctggatttgttcagaacgctcggttgccgccgggcgttttttattggtgagaatccaagcagtagtcaggatcctcaagtcggccgcccgttccatggatactcgtcgaccattacgctagccgtctggagctcggactgcttaagtcgctccatatgctcgttcccgggactacacaattgtcccccggcgccagggttgatatctatcgccctagggaccgtctcgagagaatcaatattaatccaacgcgtggcatcaaataaaacgaaaggctcagtcgaaagactgggcctttcgttttatctgttgtttgtcggtgaacgctctcctgagtaggacaaatccgccgccctagacttaggcgttcggctgcggcgagcggtatcagctcactcaaaggcggtaatacggttatccacagaatcaggggataacgcaggaaagaacatgtgagcaaaaggccagcaaaaggccaggaaccgtaaaaaggccgcgttgctggcgtttttccataggctccgcccccctgacgagcatcacaaaaatcgacgctcaagtcagaggtggcgaaacccgacaggactataaagataccaggcgtttccccctggaagctccctcgtgcgctctcctgttccgaccctgccgcttaccggatacctgtccgcctttctcccttcgggaagcgtggcgctttctcatagctcacgctgtaggtatctcagttcggtgtaggtcgttcgctccaagctgggctgtctgcacgaaccccccgttcagcccgaccgctgcgccttatccggtaactatcgtcttgagtccaacccggtaagacacgacttatcgccactggcagcagccactggtaacaggattagcagagcgaggtatgtaggcggtgctacagagttcttgaagtggtggcctaactacggctacactagaaggacagtatttggtatctgcgctctgctgaagccagttaccttcggaaaaagagttggtagctcttgatccggcaaacaaaccaccgctggtagcggtggtttttttgtttgcaagcagcagattacgcgcagaaaaaaaggatctcaagaagatcctttgatcttttctacggggtctgacgctcagtggaacgaaaactcacgttaagggattttggtcatggctagtgcttggattctcaccaataaaaaacgcccggcggcaaccgagcgttctgaacaaatccagatggagttctgaggtcattactggatctatcaacaggagtccaagccaattctcgaaccccagagtcccgctcagaagaactcgtcaagaaggcgatagaaggcgatgcgctgcgaatcgggagcggcgataccgtaaagcacgaggaagcggtcagcccattcgccgccaagctcttcagcaatatcacgggtagccaacgctatgtcctgatagcggtccgccacacccagccggccacagtcgatgaatccagaaaagcggccattttccaccatgatattcggcaagcaggcatcgccgtgggtcacgacgagatcctcgccgtcgggcatacgcgccttgagcctggcgaacagttcggctggcgcgagcccctgatgctcttcgtccagatcatcctgatcgacaagaccggcttccatccgagtacgtgctcgctcgatgcgatgtttcgcttggtggtcgaatgggcaggtagccggatcaagcgtatgcagccgccgcattgcatcagccatgatggatactttctcggcaggagcaaggtgagatgacaggagatcctgccccggcacttcgcccaatagcagccagtcccttcccgcttcagtgacaacgtcgagcacagccgcgcaaggaacgcccgtcgtggccagccacgatagccgcgctgcctcgtcttgcagttcattcagggcaccggacaggtcggtcttgacaaaaagaaccgggcgaccctgcgctgacagccggaacacggcggcatcagagcagccgattgtctgttgtgcccagtcatagccgaatagcctctccacccaagccgccggagaacctgcgtgcaatccatcttgttcaatcatgcgaaacgatcctcatcctgtctcttgatcagatcttgatcccctgcgccatcagatccttggcggcaagaaagccatccagtttactttgcagggcttcccaaccttaccagagggcggcccaactggcaattcc

SEQ ID NO: 2 - DNA, 6037 bp, Artificial Sequence
  Synthetic Polynucleotide
gacgtctgtgcaagtactactgttctgcagtcacttgaattctccctatcagtgatagagattgacatccctatcagtgatagagatactgagcacatcagcaggacgcactgacccagctgaaaagcttacgggaggaacgttatgaatcagaccgacacatcacctatcaggctgcgcaggagctggaacaccagcgagatagaagcgctctttgacgagcatgccggacgtatcgatccgcgcatttataccgatgaggatctgtaccaactcgaactggagcgtgtcttcgcccggtcctggctgctgttggggcatgaaacccagattcgcaagccgggcgattacatcacgacctacatgggtgaagaccctgtcgtggtcgtccggcagaaagacgccagcattgccgtgttcctgaaccagtgccgccaccgtggcatgcgcatctgccgcgcggatgccggaaacgcgaaggcgttcacttgcagctaccacgggtgggcttacgacaccgccggcaatcttgtcaatgtgccttacgaggccgaatccttcgcgtgcctgaacaagaaggaatggagcccgctgaaggcccgggtagaaacctacaagggcctgattttcgccaactgggatgagaacgctgtagacctcgacacgtatctgggcgaggcgaagttctacatggaccacatgctcgaccgcaccgaggccggcaccgaagcgatcccgggcgtgcagaagtgggtcattccctgtaactggaaattcgccgcagagcagttttgcagcgacatgtaccatgccgggacgacctcgcatctgtctggcatcctggcaggcctgccagaagaccttgaaatggccgaccttgctccgccgacagttggcaagcagtaccgtgcgtcatggggcggacatggaagtggcttctatgtcggcgaccccaatctgatgcttgccatcatggggccaaaggtcaccagctactggaccgaaggccccgcgtcggaaaaggcggccgaacgtctgggtagcgtggagcgcggctcgaaactcatggtcgagcacatgaccgtcttccccacgtgttccttcctcccaggtatcaatacggtccggacatggcatccgcgcgggccgaacgaggtcgaggtatgggcgtttacggtggtcgatgctgatgctcctgacgatatcaaggaagagttccggcgccagacgctgcgcaccttctctgccggtggcgtgttcgagcaggacgacggggagaactgggtcgagatccagcacatcctgcgaggccacaaggcgcggagccgccctttcaatgccgagatgagcatggaccagaccgtcgacaacgacccggtttaccccgggcggatcagcaacaacgtctacagcgaggaagctgcccgcgggctctatgcccattggctgcggatgatgacatcccccgactgggacgcgctgaaggcgacacgctgaatccagagacagcttgcgccacgcagtggcgccggccagaggccgcatttgacttcgacccaggttggatgcggtggaccttgtccatttgaaatctacaaggaacgaccatgattgattcagccaacagagccgacgtctttctccgcaagccggcacccgtagcgcccgaactgcagcacgaagtcgagcagttctactattgggaggccaagcttctcaacgatcgccgcttcgaggagtggttcgcgctgctcgcggaagacattcactacttcatgcccattcgcaccacgcggatcatgcgggactcgcgccttgaatactcaggctcccgagagtacgcgcacttcgatgacgacgccacgatgatgaagggacgcttgcgcaagatcacgtccgacgtgagctggtccgagaaccccgcatcgcggacccggcatctcgtgagcaacgtgatgatcgtcggcgcagaggcagaaggggagtacgaaatctcaagcgccttcattgtgtaccgcaatcgtctggagcggcagctcgacatctttgccggtgagcgtcgcgatacgttgcgccgtaacacgagcgaggccgggttcgagatcgtcaatcggaccatcctgatcgaccagagcaccatcctggccaataacctcagtttcttcttctaggtgatgtcatgacttggacatacatattgcggcagggtgacctgccacccggtgagatgcagcgctacgaaggcggcccggaacctgtgatggtctgcaacgtcgatggcgagttcttcgcggtgcaggatacctgcacgcatggggactgggcgttgtcggatggttacctggacggtgatattgtcgaatgcacgttgcatttcggcaagttctgcgtgcggaccgggaaggtgaaggcgctgcctgcttgcaaacctatcaaggtattcccaatcaaggtcgaaggcgatgaagtgcacgtcgatctcgacaacggggagttgaagtgatggctacccatgtggcgatcatcggcaatggcgtgggtggcttcacgaccgcgcaggccctacgtgccgagggcttcgaggggagaatctcgctgattggggacgaaccgcatctcccctatgaccgaccatccttgtccaaggcggttctcgacggcagccttgagcggccgcccatactggccgaggccgattggtacggcgaggcccgcatcgacatgctgaccggcccggaagtcactgcccttgatgtgcagacaaggacgatcagtctggatgatggcaccacgctctctgcggacgccatcgtcatcgcgacgggcagtcgagcgcggacgatggcgttgcccggcagccaactgccgggcgtcgtaacgctgcgcacctacggtgacgtgcaggtattgcgcgatagttggacttccgcgacgcggctgctgattgtgggtggcggattgatcggctgcgaggtcgcgacgacggcgcgcaagctcggcctgtcggtcacgatcctggaggcaggtgatgaactgctggtccgagtacttgggcggcgtatcggtgcctggctgcgcggcctgctgacagaacttggtgtgcaggtcgagttgggaacgggtgtcgtaggtttttctggtgagggccagctcgaacaagtcatggccagcgatgggcgcagcttcgtagccgatagcgcactcatttgcgtcggcgcggagcccgcggatcaacttgcgcgtcaagcgggcttggcatgtgaccgcggcgtcattgtcgatcactgcggtgcgacgcttgccaaaggcgtattcgccgtcggagatgtggccagttggccgctgcgcgccggcggccggcgttcgctcgaaacctatatgaacgcgcagcgccaagccgccgcggtggctgcggccattctggggaaaaacgtatcggcaccgcaactgcccgtgtcctggacggagatcgctgggcatcgcatgcagatggcgggcgatatcgaaggacctggtgatttcgtctcgcgcggcatgcccggtagtggcgctgccctgttgttccgcctgcaggagcgaaggattcaggcggtcgtcgcggtcgatgcaccccgtgacttcgcgcttgcaacccgattggtagaagcccgcgcggcaatcgagccagcacggctggcagatctttcaaacagtatgcgcgattttgttcgtgcgaatgaaggagacctaacgtgaggtacccgagaattggcttggactcctgttgatagatccagtaatgacctcagaactccatctggatttgttcagaacgctcggttgccgccgggcgttttttattggtgagaatccaagcagtagtcaggatcctcaagtcggccgcccgttccatggatactcgtcgaccattacgctagccgtctggagctcggactgcttaagtcgctccatatgctcgttcccgggactacacaattgtcccccggcgccagggttgatatctatcgccctagggaccgtctcgagagaatcaatattaatccaacgcgtggcatcaaataaaacgaaaggctcagtcgaaagactgggcctttcgttttatctgttgtttgtcggtgaacgctctcctgagtaggacaaatccgccgccctagacttaggcgttcggctgcggcgagcggtatcagctcactcaaaggcggtaatacggttatccacagaatcaggggataacgcaggaaagaacatgtgagcaaaaggccagcaaaaggccaggaaccgtaaaaaggccgcgttgctggcgtttttccataggctccgcccccctgacgagcatcacaaaaatcgacgctcaagtcagaggtggcgaaacccgacaggactataaagataccaggcgtttccccctggaagctccctcgtgcgctctcctgttccgaccctgccgcttaccggatacctgtccgcctttctcccttcgggaagcgtggcgctttctcatagctcacgctgtaggtatctcagttcggtgtaggtcgttcgctccaagctgggctgtctgcacgaaccccccgttcagcccgaccgctgcgccttatccggtaactatcgtcttgagtccaacccggtaagacacgacttatcgccactggcagcagccactggtaacaggattagcagagcgaggtatgtaggcggtgctacagagttcttgaagtggtggcctaactacggctacactagaaggacagtatttggtatctgcgctctgctgaagccagttaccttcggaaaaagagttggtagctcttgatccggcaaacaaaccaccgctggtagcggtggtttttttgtttgcaagcagcagattacgcgcagaaaaaaaggatctcaagaagatcctttgatcttttctacggggtctgacgctcagtggaacgaaaactcacgttaagggattttggtcatggctagtgcttggattctcaccaataaaaaacgcccggcggcaaccgagcgttctgaacaaatccagatggagttctgaggtcattactggatctatcaacaggagtccaagccaattctcgaaccccagagtcccgctcagaagaactcgtcaagaaggcgatagaaggcgatgcgctgcgaatcgggagcggcgataccgtaaagcacgaggaagcggtcagcccattcgccgccaagctcttcagcaatatcacgggtagccaacgctatgtcctgatagcggtccgccacacccagccggccacagtcgatgaatccagaaaagcggccattttccaccatgatattcggcaagcaggcatcgccgtgggtcacgacgagatcctcgccgtcgggcatacgcgccttgagcctggcgaacagttcggctggcgcgagcccctgatgctcttcgtccagatcatcctgatcgacaagaccggcttccatccgagtacgtgctcgctcgatgcgatgtttcgcttggtggtcgaatgggcaggtagccggatcaagcgtatgcagccgccgcattgcatcagccatgatggatactttctcggcaggagcaaggtgagatgacaggagatcctgccccggcacttcgcccaatagcagccagtcccttcccgcttcagtgacaacgtcgagcacagccgcgcaaggaacgcccgtcgtggccagccacgatagccgcgctgcctcgtcttgcagttcattcagggcaccggacaggtcggtcttgacaaaaagaaccgggcgaccctgcgctgacagccggaacacggcggcatcagagcagccgattgtctgttgtgcccagtcatagccgaatagcctctccacccaagccgccggagaacctgcgtgcaatccatcttgttcaatcatgcgaaacgatcctcatcctgtctcttgatcagatcttgatcccctgcgccatcagatccttggcggcaagaaagccatccagtttactttgcagggcttcccaaccttaccagagggcggcccaactggcaattcc

SEQ ID NO: 3 - DNA, 4497 bp, Artificial Sequence
  Synthetic Polynucleotide
gacgtctgtgcaagtactaagaaaccaatagtccatattgcatcagacattgccgtcactgcgtcttttactggctcttctcgctaaccaaaccggtaaccccgcttattaaaagcattctgtaacaaagcgggaccaaagccatgacaaaagcgcgtaacaaaagtgtctataatcacggcagaaaagtccacattgattatttgcacggcgtcacactttgctatgccatagcatttttatccataagattagcggatcatacctgacgctttttatcgcaactctctactgtttctccatacagctgaaggattaaggaggtagcatgcatgaaaaagcgtatcggtattgttggtgcaggcactgccggcctccatcttggcctcttcctccgccagcatgacgtcgacgtcactgtgtacactgatcgtaagcccgatgagtacagtggactgcggctcctgaataccgttgctcacaacgcggtgacggtgcagcgggaggttgccctcgacgtcaatgagtggccgtctgaggagtttggctatttcggccactactactacgtaggtgggccgcagcccatgcgtttctacggtgatctcaaggctcccagccgtgcagtggactaccgtctctacctgccgatgctgatgcgtgcactggaagccaggggcggcaagttctgctacgacgccgtgtctgccgaagatctggaagggctgtcggagcagtatgatctgctggttgtgtgcactggtaaatacgccctcggcaaggtgttcgagaagcagtccgaaaactcgcccttcgagaagccgcaacgggcactgtgcgttggtctcttcaagggcatcaaggaagcaccgattcgcgcggtgactatgtccttctcgccagggcatggcgagctgattgagattccaaccctgtcgttcaatggcatgagcacagcgctggtgctcgaaaaccatattggtagcgatctggaagtcctcgcccacaccaagtatgacgatgacccgcgtgcgttcctcgatctgatgctggagaagctgcgtaagcatcatccttccgttgccgagcgcatcgatccggctgagttcgacctggccaacagttctctggacatcctccagggcggtgttgtgccagtattccgcgacggtcatgcgaccctcaataacggcaaaaccatcatcgggctgggcgacatccaggcaactgtcgatccggtcttgggccagggcgcgaacatggcgtcctatgcggcatggattctgggcgaggaaatccttgcgcactctgtctacgacctgcgcttcagcgaacacctggagcgtcgccgccaggatcgcgtgctgtgcgccacccgctggaccaacttcactctgagcgccttcacggaacttccgccggaattcctcaccttccttcagatcctgagccagagccgtgaaatggctgatgagttcacggacaacttcaactatccggaacttcagtgggatcgcttctccagcccggaacgtatcggtcagtggtgcagccagtacgcacccactattgcggcctgacgctattgctccgctggtcaaggccagcggagccctaactcctgggtgattcaaatgacgttaaaaaaagatgtggtggtggatatcgactccaccagcttccgccaggcggttgcactgttcgcgacgggaattgcggttctcagcgcggagactgacgagggcgaagtgcatggcatgacggtgaacagcttcacctccatcagtctggacccgccgactgtgatggtgtccctgaagtcgggccgtatgcatgagctgctgactcaaggcggacgcttcggcgtcagcctcctgggtgaaagtcagaagatgttatcggcattcttcagcaagcgtgtgatcgatggcactcctcctcctgctttcacagttcaggccggcctccccactctgcgggacgccatggcctggttcgaatgcgaggtggagagcacggttgaagtacacgaccacacgctcttcattgcgcgcgttagcgcctgtggagtgccggaggcgaatgccccccagccgctgctgttctttgccagccgttatcacggcaacccgttgccgctgaattgaaacgttcgagaattggcttggactcctgttgatagatccagtaatgacctcagaactccatctggatttgttcagaacgctcggttgccgccgggcgttttttattggtgagaatccaagcagtagtcaaagcttccgcaaggtaccactttgccgcggagtatttgtacatttgaaggatcctcaagtcggccgcccgttccatggatactcgtcgaccattacgctagccgtctggagctcggactgcttaagtcgctccatatgctcgttcccgggactacacaattgtcccccggcgccagggttgatatctatcgccctagggaccgtctcgagagaatcaatattaatccaacgcgtggcatcaaataaaacgaaaggctcagtcgaaagactgggcctttcgttttatctgttgtttgtcggtgaacgctctcctgagtaggacaaatccgccgccctagacttaggcgttcggctgcggcgagcggtatcagctcactcaaaggcggtaatacggttatccacagaatcaggggataacgcaggaaagaacatgtgagcaaaaggccagcaaaaggccaggaaccgtaaaaaggccgcgttgctggcgtttttccataggctccgcccccctgacgagcatcacaaaaatcgacgctcaagtcagaggtggcgaaacccgacaggactataaagataccaggcgtttccccctggaagctccctcgtgcgctctcctgttccgaccctgccgcttaccggatacctgtccgcctttctcccttcgggaagcgtggcgctttctcatagctcacgctgtaggtatctcagttcggtgtaggtcgttcgctccaagctgggctgtctgcacgaaccccccgttcagcccgaccgctgcgccttatccggtaactatcgtcttgagtccaacccggtaagacacgacttatcgccactggcagcagccactggtaacaggattagcagagcgaggtatgtaggcggtgctacagagttcttgaagtggtggcctaactacggctacactagaaggacagtatttggtatctgcgctctgctgaagccagttaccttcggaaaaagagttggtagctcttgatccggcaaacaaaccaccgctggtagcggtggtttttttgtttgcaagcagcagattacgcgcagaaaaaaaggatctcaagaagatcctttgatcttttctacggggtctgacgctcagtggaacgaaaactcacgttaagggattttggtcatggctagtgcttggattctcaccaataaaaaacgcccggcggcaaccgagcgttctgaacaaatccagatggagttctgaggtcattactggatctatcaacaggagtccaagccaattctcgaaccccagagtcccgctcagaagaactcgtcaagaaggcgatagaaggcgatgcgctgcgaatcgggagcggcgataccgtaaagcacgaggaagcggtcagcccattcgccgccaagctcttcagcaatatcacgggtagccaacgctatgtcctgatagcggtccgccacacccagccggccacagtcgatgaatccagaaaagcggccattttccaccatgatattcggcaagcaggcatcgccgtgggtcacgacgagatcctcgccgtcgggcatacgcgccttgagcctggcgaacagttcggctggcgcgagcccctgatgctcttcgtccagatcatcctgatcgacaagaccggcttccatccgagtacgtgctcgctcgatgcgatgtttcgcttggtggtcgaatgggcaggtagccggatcaagcgtatgcagccgccgcattgcatcagccatgatggatactttctcggcaggagcaaggtgagatgacaggagatcctgccccggcacttcgcccaatagcagccagtcccttcccgcttcagtgacaacgtcgagcacagccgcgcaaggaacgcccgtcgtggccagccacgatagccgcgctgcctcgtcttgcagttcattcagggcaccggacaggtcggtcttgacaaaaagaaccgggcgaccctgcgctgacagccggaacacggcggcatcagagcagccgattgtctgttgtgcccagtcatagccgaatagcctctccacccaagccgccggagaacctgcgtgcaatccatcttgttcaatcatgcgaaacgatcctcatcctgtctcttgatcagatcttgatcccctgcgccatcagatccttggcggcaagaaagccatccagtttactttgcagggcttcccaaccttaccagagggcggcccaactggcaattcc

SEQ ID NO: 4 - DNA, 4285 bp, Artificial Sequence
  Synthetic Polynucleotide
gacgtctgtgcaagtacttccctatcagtgatagagattgacatccctatcagtgatagagatactgagcacatcagcaggacgcactgacccagctgaaggattaaggaggtagcatgcatgaaaaagcgtatcggtattgttggtgcaggcactgccggcctccatcttggcctcttcctccgccagcatgacgtcgacgtcactgtgtacactgatcgtaagcccgatgagtacagtggactgcggctcctgaataccgttgctcacaacgcggtgacggtgcagcgggaggttgccctcgacgtcaatgagtggccgtctgaggagtttggctatttcggccactactactacgtaggtgggccgcagcccatgcgtttctacggtgatctcaaggctcccagccgtgcagtggactaccgtctctacctgccgatgctgatgcgtgcactggaagccaggggcggcaagttctgctacgacgccgtgtctgccgaagatctggaagggctgtcggagcagtatgatctgctggttgtgtgcactggtaaatacgccctcggcaaggtgttcgagaagcagtccgaaaactcgcccttcgagaagccgcaacgggcactgtgcgttggtctcttcaagggcatcaaggaagcaccgattcgcgcggtgactatgtccttctcgccagggcatggcgagctgattgagattccaaccctgtcgttcaatggcatgagcacagcgctggtgctcgaaaaccatattggtagcgatctggaagtcctcgcccacaccaagtatgacgatgacccgcgtgcgttcctcgatctgatgctggagaagctgcgtaagcatcatccttccgttgccgagcgcatcgatccggctgagttcgacctggccaacagttctctggacatcctccagggcggtgttgtgccagtattccgcgacggtcatgcgaccctcaataacggcaaaaccatcatcgggctgggcgacatccaggcaactgtcgatccggtcttgggccagggcgcgaacatggcgtcctatgcggcatggattctgggcgaggaaatccttgcgcactctgtctacgacctgcgcttcagcgaacacctggagcgtcgccgccaggatcgcgtgctgtgcgccacccgctggaccaacttcactctgagcgccttcacggaacttccgccggaattcctcaccttccttcagatcctgagccagagccgtgaaatggctgatgagttcacggacaacttcaactatccggaacttcagtgggatcgcttctccagcccggaacgtatcggtcagtggtgcagccagtacgcacccactattgcggcctgacgctattgctccgctggtcaaggccagcggagccctaactcctgggtgattcaaatgacgttaaaaaaagatgtggtggtggatatcgactccaccagcttccgccaggcggttgcactgttcgcgacgggaattgcggttctcagcgcggagactgacgagggcgaagtgcatggcatgacggtgaacagcttcacctccatcagtctggacccgccgactgtgatggtgtccctgaagtcgggccgtatgcatgagctgctgactcaaggcggacgcttcggcgtcagcctcctgggtgaaagtcagaagatgttatcggcattcttcagcaagcgtgtgatcgatggcactcctcctcctgctttcacagttcaggccggcctccccactctgcgggacgccatggcctggttcgaatgcgaggtggagagcacggttgaagtacacgaccacacgctcttcattgcgcgcgttagcgcctgtggagtgccggaggcgaatgccccccagccgctgctgttctttgccagccgttatcacggcaacccgttgccgctgaattgaaacgttcgagaattggcttggactcctgttgatagatccagtaatgacctcagaactccatctggatttgttcagaacgctcggttgccgccgggcgttttttattggtgagaatccaagcagtagtcaaagcttccgcaaggtaccactttgccgcggagtatttgtacatttgaaggatcctcaagtcggccgcccgttccatggatactcgtcgaccattacgctagccgtctggagctcggactgcttaagtcgctccatatgctcgttcccgggactacacaattgtcccccggcgccagggttgatatctatcgccctagggaccgtctcgagagaatcaatattaatccaacgcgtggcatcaaataaaacgaaaggctcagtcgaaagactgggcctttcgttttatctgttgtttgtcggtgaacgctctcctgagtaggacaaatccgccgccctagacttaggcgttcggctgcggcgagcggtatcagctcactcaaaggcggtaatacggttatccacagaatcaggggataacgcaggaaagaacatgtgagcaaaaggccagcaaaaggccaggaaccgtaaaaaggccgcgttgctggcgtttttccataggctccgcccccctgacgagcatcacaaaaatcgacgctcaagtcagaggtggcgaaacccgacaggactataaagataccaggcgtttccccctggaagctccctcgtgcgctctcctgttccgaccctgccgcttaccggatacctgtccgcctttctcccttcgggaagcgtggcgctttctcatagctcacgctgtaggtatctcagttcggtgtaggtcgttcgctccaagctgggctgtctgcacgaaccccccgttcagcccgaccgctgcgccttatccggtaactatcgtcttgagtccaacccggtaagacacgacttatcgccactggcagcagccactggtaacaggattagcagagcgaggtatgtaggcggtgctacagagttcttgaagtggtggcctaactacggctacactagaaggacagtatttggtatctgcgctctgctgaagccagttaccttcggaaaaagagttggtagctcttgatccggcaaacaaaccaccgctggtagcggtggtttttttgtttgcaagcagcagattacgcgcagaaaaaaaggatctcaagaagatcctttgatcttttctacggggtctgacgctcagtggaacgaaaactcacgttaagggattttggtcatggctagtgcttggattctcaccaataaaaaacgcccggcggcaaccgagcgttctgaacaaatccagatggagttctgaggtcattactggatctatcaacaggagtccaagccaattctcgaaccccagagtcccgctcagaagaactcgtcaagaaggcgatagaaggcgatgcgctgcgaatcgggagcggcgataccgtaaagcacgaggaagcggtcagcccattcgccgccaagctcttcagcaatatcacgggtagccaacgctatgtcctgatagcggtccgccacacccagccggccacagtcgatgaatccagaaaagcggccattttccaccatgatattcggcaagcaggcatcgccgtgggtcacgacgagatcctcgccgtcgggcatacgcgccttgagcctggcgaacagttcggctggcgcgagcccctgatgctcttcgtccagatcatcctgatcgacaagaccggcttccatccgagtacgtgctcgctcgatgcgatgtttcgcttggtggtcgaatgggcaggtagccggatcaagcgtatgcagccgccgcattgcatcagccatgatggatactttctcggcaggagcaaggtgagatgacaggagatcctgccccggcacttcgcccaatagcagccagtcccttcccgcttcagtgacaacgtcgagcacagccgcgcaaggaacgcccgtcgtggccagccacgatagccgcgctgcctcgtcttgcagttcattcagggcaccggacaggtcggtcttgacaaaaagaaccgggcgaccctgcgctgacagccggaacacggcggcatcagagcagccgattgtctgttgtgcccagtcatagccgaatagcctctccacccaagccgccggagaacctgcgtgcaatccatcttgttcaatcatgcgaaacgatcctcatcctgtctcttgatcagatcttgatcccctgcgccatcagatccttggcggcaagaaagccatccagtttactttgcagggcttcccaaccttaccagagggcggcccaactggcaattcc

SEQ ID NO: 5 - DNA, 9507 bp, Artificial Sequence
  Synthetic Polynucleotide
aatgctactactattagtagaattgatgccaccttttcagctcgcgccccaaatgaaaatatagctaaacaggttattgaccatttgcgaaatgtatctaatggtcaaactaaatctactcgttcgcagaattgggaatcaactgttatatggaatgaaacttccagacaccgtactttagttgcatatttaaaacatgttgagctacagcattatattcagcaattaagctctaagccatccgcaaaaatgacctcttatcaaaaggagcaattaaaggtactctctaatcctgacctgttggagtttgcttccggtctggttcgctttgaagctcgaattaaaacgcgatatttgaagtctttcgggcttcctcttaatctttttgatgcaatccgctttgcttctgactataatagtcagggtaaagacctgatttttgatttatggtcattctcgttttctgaactgtttaaagcatttgagggggattcaatgaatatttatgacgattccgcagtattggacgctatccagtctaaacattttactattaccccctctggcaaaacttcttttgcaaaagcctctcgctattttggtttttatcgtcgtctggtaaacgagggttatgatagtgttgctcttactatgcctcgtaattccttttggcgttatgtatctgcattagttgaatgtggtattcctaaatctcaactgatgaatctttctacctgtaataatgttgttccgttagttcgttttattaacgtagatttttcttcccaacgtcctgactggtataatgagccagttcttaaaatcgcataaggtaattcacaatgattaaagttgaaattaaaccatctcaagcccaatttactactcgttctggtgtttctcgtcagggcaagccttattcactgaatgagcagctttgttacgttgatttgggtaatgaatatccggttcttgtcaagattactcttgatgaaggtcagccagcctatgcgcctggtctgtacaccgttcatctgtcctctttcaaagttggtcagttcggttcccttatgattgaccgtctgcgcctcgttccggctaagtaacatggagcaggtcgcggatttcgacacaatttatcaggcgatgatacaaatctccgttgtactttgtttcgcgcttggtataatcgctgggggtcaaagatgagtgttttagtgtattcttttgcctctttcgttttaggttggtgccttcgtagtggcattacgtattttacccgtttaatggaaacttcctcatgaaaaagtctttagtcctcaaagcctctgtagccgttgctaccctcgttccgatgctgtctttcgctgctgagggtgacgatcccgcaaaagcggcctttaactccctgcaagcctcagcgaccgaatatatcggttatgcgtgggcgatggttgttgtcattgtcggcgcaactatcggtatcaagctgtttaagaaattcacctcgaaagcaagctgataaaccgatacaattaaaggctccttttggagccttttttttggagattttcaacgtgaaaaaattattattcgcaattcctttagttgttcctttctattctcactccgctgaaactgttgaaagttgtttagcaaaatcccatacagaaaattcatttactaacgtctggaaagacgacaaaactttagatcgttacgctaactatgagggctgtctgtggaatgctacaggcgttgtagtttgtactggtgacgaaactcagtgttacggtacatgggttcctattgggcttgctatccctgaaaatgagggtggtggctctgagggtggcggttctgagggtggcggttctgagggtggcggtactaaacctcctgagtacggtgatacacctattccgggctatacttatatcaaccctctcgacggcacttatccgcctggtactgagcaaaaccccgctaatcctaatccttctcttgaggagtctcagcctcttaatactttcatgtttcagaataataggttccgaaataggcagggggcattaactgtttatacgggcactgttactcaaggcactgaccccgttaaaacttattaccagtacactcctgtatcatcaaaagccatgtatgacgcttactggaacggtaaattcagagactgcgctttccattctggctttaatgaggatttatttgtttgtgaatatcaaggccaatcgtctgacctgcctcaacctcctgtcaatgctggcggcggctctggtggtggttctggtggcggctctgagggtggtggctctgagggtggcggttctgagggtggcggctctgagggaggcggttccggtggtggctctggttccggtgattttgattatgaaaagatggcaaacgctaataagggggctatgaccgaaaatgccgatgaaaacgcgctacagtctgacgctaaaggcaaacttgattctgtcgctactgattacggtgctgctatcgatggtttcattggtgacgtttccggccttgctaatggtaatggtgctactggtgattttgctggctctaattcccaaatggctcaagtcggtgacggtgataattcacctttaatgaataatttccgtcaatatttaccttccctccctcaatcggttgaatgtcgcccttttgtctttggcgctggtaaaccatatgaattttctattgattgtgacaaaataaacttattccgtggtgtctttgcgtttcttttatatgttgccacctttatgtatgtattttctacgtttgctaacatactgcgtaataaggagtcttaatcatgccagttcttttgggtattccgttattattgcgtttcctcggtttccttctggtaactttgttcggctatctgcttacttttcttaaaaagggcttcggtaagatagctattgctatttcattgtttcttgctcttattattgggcttaactcaattcttgtgggttatctctctgatattagcgctcaattaccctctgactttgttcagggtgttcagttaattctcccgtctaatgcgcttccctgtttttatgttattctctctgtaaaggctgctattttcatttttgacgttaaacaaaaaatcgtttcttatttggattgggataaataatatggctgtttattttgtaactggcaaattaggctctggaaagacgctcgttagcgttggtaagattcaggataaaattgtagctgggtgcaaaatagcaactaatcttgatttaaggcttcaaaacctcccgcaagtcgggaggttcgctaaaacgcctcgcgttcttagaataccggataagccttctatatctgatttgcttgctattgggcgcggtaatgattcctacgatgaaaataaaaacggcttgcttgttctcgatgagtgcggtacttggtttaatacccgttcttggaatgataaggaaagacagccgattattgattggtttctacatgctcgtaaattaggatgggatattatttttcttgttcaggacttatctattgttgataaacaggcgcgttctgcattagctgaacatgttgtttattgtcgtcgtctggacagaattactttaccttttgtcggtactttatattctcttattactggctcgaaaatgcctctgcctaaattacatgttggcgttgttaaatatggcgattctcaattaagccctactgttgagcgttggctttatactggtaagaatttgtataacgcatatgatactaaacaggctttttctagtaattatgattccggtgtttattcttatttaacgccttatttatcacacggtcggtatttcaaaccattaaatttaggtcagaagatgaaattaactaaaatatatttgaaaaagttttctcgcgttctttgtcttgcgattggatttgcatcagcatttacatatagttatataacccaacctaagccggaggttaaaaaggtagtctctcagacctatgattttgataaattcactattgactcttctcagcgtcttaatctaagctatcgctatgttttcaaggattctaagggaaaattaattaatagcgacgatttacagaagcaaggttattcactcacatatattgatttatgtactgtttccattaaaaaaggtaattcaaatgaaattgttaaatgtaattaattttgttttcttgatgtttgtttcatcatcttcttttgctcaggtaattgaaatgaataattcgcctctgcgcgattttgtaacttggtattcaaagcaatcaggcgaatccgttattgtttctcccgatgtaaaaggtactgttactgtatattcatctgacgttaaacctgaaaatctacgcaatttctttatttctgttttacgtgcaaataattttgatatggtaggttctaacccttccattattcagaagtataatccaaacaatcaggattatattgatgaattgccatcatctgataatcaggaatatgatgataattccgctccttctggtggtttctttgttccgcaaaatgataatgttactcaaacttttaaaattaataacgttcgggcaaaggatttaatacgagttgtcgaattgtttgtaaagtctaatacttctaaatcctcaaatgtattatctattgacggctctaatctattagttgttagtgctcctaaagatattttagataaccttcctcaattcctttcaactgttgatttgccaactgaccagatattgattgagggtttgatatttgaggttcagcaaggtgatgctttagatttttcatttgctgctggctctcagcgtggcactgttgcaggcggtgttaatactgaccgcctcacctctgttttatcttctgctggtggttcgttcggtatttttaatggcgatgttttagggctatcagttcgcgcattaaagactaatagccattcaaaaatattgtctgtgccacgtattcttacgctttcaggtcagaagggttctatctctgttggccagaatgtcccttttattactggtcgtgtgactggtgaatctgccaatgtaaataatccatttcagacgattgagcgtcaaaatgtaggtatttccatgagcgtttttcctgttgcaatggctggcggtaatattgttctggatattaccagcaaggccgatagtttgagttcttctactcaggcaagtgatgttattactaatcaaagaagtattgctacaacggttaatttgcgtgatggacagactcttttactcggtggcctcactgattataaaaacacttctcaggattctggcgtaccgttcctgtctaaaatccctttaatcggcctcctgtttagctcccgctctgattctaacgaggaaagcacgttatacgtgctcgtcaaagcaaccatagtacgcgccctgtagcggcgcattaagcgcggcgggtgtggtggttacgcgcagcgtgaccgctacacttgccagcgccctagcgcccgctcctttcgctttcttcccttcctttctcgccacgttcgccggctttccccgtcaagctctaaatcgggggctccctttagggttccgatttagtgctttacggcacctcgaccccaaaaaacttgatttgggtgatggttcacgtagtgggccatcgccctgatagacggtttttcgccctttgacgttggagtccacgttctttaatagtggactcttgttccaaactggaacaacactcaaccctatctcgggctattcttttgatttataagggattttgccgatttcggaaccaccatcaaacaggattttcgcctgctggggcaaaccagcgtggaccgcttgctgcaactctctcagggccaggcggtgaagggcaatcagctgttgcccgtctcactggtgaaaagaaaaaccaccctggcgcccaatacgcaaaccgcctctccccgcgcgttggccgattcattaatgcagctggcacgacaggtttcccgactggaaagcgggcagtgagcgcaacgcaattaatgtgagttagctcactcattaggcaccccaggctttacactttatgcttccggctcgtatgttgtgtggaattgtgagcggataacaatttcacacaggaaacagctatgaccatgattacgaattcgagctctgactactgcttggattctcaccaataaaaaacgcccggcggcaaccgagcgttctgaacaaatccagatggagttctgaggtcattactggatctatcaacaggagtccaagccaattctcgaacgtttcaattcagcggcaacgggttgccgtgataacggctggcaaagaacagcagcggctggggggcattcgcctccggcactccacaggcgctaacgcgcgcaatgaagagcgtgtggtcgtgtacttcaaccgtgctctccacctcgcattcgaaccaggccatggcgtcccgcagagtggggaggccggcctgaactgtgaaagcaggaggaggagtgccatcgatcacacgcttgctgaagaatgccgataacatcttctgactttcacccaggaggctgacgccgaagcgtccgccttgagtcagcagctcatgcatacggcccgacttcagggacaccatcacagtcggcgggtccagactgatggaggtgaagctgttcaccgtcatgccatgcacttcgccctcgtcagtctccgcgctgagaaccgcaattcccgtcgcgaacagtgcaaccgcctggcggaagctggtggagtcgatatccaccaccacatctttttttaacgtcatttgaatcacccaggagttagggctccgctggccttgaccagcggagcaatagcgtcaggccgcaatagtgggtgcgtactggctgcaccactgaccgatacgttccgggctggagaagcgatcccactgaagttccggatagttgaagttgtccgtgaactcatcagccatttcacggctctggctcaggatctgaaggaaggtgaggaattccggcggaagttccgtgaaggcgctcagagtgaagttggtccagcgggtggcgcacagcacgcgatcctggcggcgacgctccaggtgttcgctgaagcgcaggtcgtagacagagtgcgcaaggatttcctcgcccagaatccatgccgcataggacgccatgttcgcgccctggcccaagaccggatcgacagttgcctggatgtcgcccagcccgatgatggttttgccgttattgagggtcgcatgaccgtcgcggaatactggcacaacaccgccctggaggatgtccagagaactgttggccaggtcgaactcagccggatcgatgcgctcggcaacggaaggatgatgcttacgcagcttctccagcatcagatcgaggaacgcacgcgggtcatcgtcatacttggtgtgggcgaggacttccagatcgctaccaatatggttttcgagcaccagcgctgtgctcatgccattgaacgacagggttggaatctcaatcagctcgccatgccctggcgagaaggacatagtcaccgcgcgaatcggtgcttccttgatgcccttgaagagaccaacgcacagtgcccgttgcggcttctcgaagggcgagttttcggactgcttctcgaacaccttgccgagggcgtatttaccagtgcacacaaccagcagatcatactgctccgacagcccttccagatcttcggcagacacggcgtcgtagcagaacttgccgcccctggcttccagtgcacgcatcagcatcggcaggtagagacggtagtccactgcacggctgggagccttgagatcaccgtagaaacgcatgggctgcggcccacctacgtagtagtagtggccgaaatagccaaactcctcagacggccactcattgacgtcgagggcaacctcccgctgcaccgtcaccgcgttgtgagcaacggtattcaggagccgcagtccactgtactcatcgggcttacgatcagtgtacacagtgacgtcgacgtcatgctggcggaggaagaggccaagatggaggccggcagtgcctgcaccaacaataccgatacgctttttcatgcatgctacctccttaatccttcagctgtatggagaaacagtagagagttgcgataaaaagcgtcaggtatgatccgctaatcttatggataaaaatgctatggcatagcaaagtgtgacgccgtgcaaataatcaatgtggacttttctgccgtgattatagacacttttgttacgcgcttttgtcatggctttggtcccgctttgttacagaatgcttttaataagcggggttaccggtttggttagcgagaagagccagtaaaagacgcagtgacggcaatgtctgatgcaatatggactattggtttcttggtacccggggatcctctagagtcgacctgcaggcatgcaagcttggcactggccgtcgttttacaacgtcgtgactgggaaaaccctggcgttacccaacttaatcgccttgcagcacatccccctttcgccagctggcgtaatagcgaagaggcccgcaccgatcgcccttcccaacagttgcgcagcctgaatggcgaatggcgctttgcctggtttccggcaccagaagcggtgccggaaagctggctggagtgcgatcttcctgaggccgatactgtcgtcgtcccctcaaactggcagatgcacggttacgatgcgcccatctacaccaacgtgacctatcccattacggtcaatccgccgtttgttcccacggagaatccgacgggttgttactcgctcacatttaatgttgatgaaagctggctacaggaaggccagacgcgaattatttttgatggcgttcctattggttaaaaaatgagctgatttaacaaaaatttaatgcgaattttaacaaaatattaacgtttacaatttaaatatttgcttatacaatcttcctgtttttggggcttttctgattatcaaccggggtacatatgattgacatgctagttttacgattaccgttcatcgattctcttgtttgctccagactctcaggcaatgacctgatagcctttgtagatctctcaaaaatagctaccctctccggcattaatttatcagctagaacggttgaatatcatattgatggtgatttgactgtctccggcctttctcacccttttgaatctttacctacacattactcaggcattgcatttaaaatatatgagggttctaaaaatttttatccttgcgttgaaataaaggcttctcccgcaaaagtattacagggtcataatgtttttggtacaaccgatttagctttatgctctgaggctttattgcttaattttgctaattctttgccttgcctgtatgatttattggatgtt

SEQ ID NO: 6 - DNA, 9295 bp, Artificial Sequence
  Synthetic Polynucleotide
aatgctactactattagtagaattgatgccaccttttcagctcgcgccccaaatgaaaatatagctaaacaggttattgaccatttgcgaaatgtatctaatggtcaaactaaatctactcgttcgcagaattgggaatcaactgttatatggaatgaaacttccagacaccgtactttagttgcatatttaaaacatgttgagctacagcattatattcagcaattaagctctaagccatccgcaaaaatgacctcttatcaaaaggagcaattaaaggtactctctaatcctgacctgttggagtttgcttccggtctggttcgctttgaagctcgaattaaaacgcgatatttgaagtctttcgggcttcctcttaatctttttgatgcaatccgctttgcttctgactataatagtcagggtaaagacctgatttttgatttatggtcattctcgttttctgaactgtttaaagcatttgagggggattcaatgaatatttatgacgattccgcagtattggacgctatccagtctaaacattttactattaccccctctggcaaaacttcttttgcaaaagcctctcgctattttggtttttatcgtcgtctggtaaacgagggttatgatagtgttgctcttactatgcctcgtaattccttttggcgttatgtatctgcattagttgaatgtggtattcctaaatctcaactgatgaatctttctacctgtaataatgttgttccgttagttcgttttattaacgtagatttttcttcccaacgtcctgactggtataatgagccagttcttaaaatcgcataaggtaattcacaatgattaaagttgaaattaaaccatctcaagcccaatttactactcgttctggtgtttctcgtcagggcaagccttattcactgaatgagcagctttgttacgttgatttgggtaatgaatatccggttcttgtcaagattactcttgatgaaggtcagccagcctatgcgcctggtctgtacaccgttcatctgtcctctttcaaagttggtcagttcggttcccttatgattgaccgtctgcgcctcgttccggctaagtaacatggagcaggtcgcggatttcgacacaatttatcaggcgatgatacaaatctccgttgtactttgtttcgcgcttggtataatcgctgggggtcaaagatgagtgttttagtgtattcttttgcctctttcgttttaggttggtgccttcgtagtggcattacgtattttacccgtttaatggaaacttcctcatgaaaaagtctttagtcctcaaagcctctgtagccgttgctaccctcgttccgatgctgtctttcgctgctgagggtgacgatcccgcaaaagcggcctttaactccctgcaagcctcagcgaccgaatatatcggttatgcgtgggcgatggttgttgtcattgtcggcgcaactatcggtatcaagctgtttaagaaattcacctcgaaagcaagctgataaaccgatacaattaaaggctccttttggagccttttttttggagattttcaacgtgaaaaaattattattcgcaattcctttagttgttcctttctattctcactccgctgaaactgttgaaagttgtttagcaaaatcccatacagaaaattcatttactaacgtctggaaagacgacaaaactttagatcgttacgctaactatgagggctgtctgtggaatgctacaggcgttgtagtttgtactggtgacgaaactcagtgttacggtacatgggttcctattgggcttgctatccctgaaaatgagggtggtggctctgagggtggcggttctgagggtggcggttctgagggtggcggtactaaacctcctgagtacggtgatacacctattccgggctatacttatatcaaccctctcgacggcacttatccgcctggtactgagcaaaaccccgctaatcctaatccttctcttgaggagtctcagcctcttaatactttcatgtttcagaataataggttccgaaataggcagggggcattaactgtttatacgggcactgttactcaaggcactgaccccgttaaaacttattaccagtacactcctgtatcatcaaaagccatgtatgacgcttactggaacggtaaattcagagactgcgctttccattctggctttaatgaggatttatttgtttgtgaatatcaaggccaatcgtctgacctgcctcaacctcctgtcaatgctggcggcggctctggtggtggttctggtggcggctctgagggtggtggctctgagggtggcggttctgagggtggcggctctgagggaggcggttccggtggtggctctggttccggtgattttgattatgaaaagatggcaaacgctaataagggggctatgaccgaaaatgccgatgaaaacgcgctacagtctgacgctaaaggcaaacttgattctgtcgctactgattacggtgctgctatcgatggtttcattggtgacgtttccggccttgctaatggtaatggtgctactggtgattttgctggctctaattcccaaatggctcaagtcggtgacggtgataattcacctttaatgaataatttccgtcaatatttaccttccctccctcaatcggttgaatgtcgcccttttgtctttggcgctggtaaaccatatgaattttctattgattgtgacaaaataaacttattccgtggtgtctttgcgtttcttttatatgttgccacctttatgtatgtattttctacgtttgctaacatactgcgtaataaggagtcttaatcatgccagttcttttgggtattccgttattattgcgtttcctcggtttccttctggtaactttgttcggctatctgcttacttttcttaaaaagggcttcggtaagatagctattgctatttcattgtttcttgctcttattattgggcttaactcaattcttgtgggttatctctctgatattagcgctcaattaccctctgactttgttcagggtgttcagttaattctcccgtctaatgcgcttccctgtttttatgttattctctctgtaaaggctgctattttcatttttgacgttaaacaaaaaatcgtttcttatttggattgggataaataatatggctgtttattttgtaactggcaaattaggctctggaaagacgctcgttagcgttggtaagattcaggataaaattgtagctgggtgcaaaatagcaactaatcttgatttaaggcttcaaaacctcccgcaagtcgggaggttcgctaaaacgcctcgcgttcttagaataccggataagccttctatatctgatttgcttgctattgggcgcggtaatgattcctacgatgaaaataaaaacggcttgcttgttctcgatgagtgcggtacttggtttaatacccgttcttggaatgataaggaaagacagccgattattgattggtttctacatgctcgtaaattaggatgggatattatttttcttgttcaggacttatctattgttgataaacaggcgcgttctgcattagctgaacatgttgtttattgtcgtcgtctggacagaattactttaccttttgtcggtactttatattctcttattactggctcgaaaatgcctctgcctaaattacatgttggcgttgttaaatatggcgattctcaattaagccctactgttgagcgttggctttatactggtaagaatttgtataacgcatatgatactaaacaggctttttctagtaattatgattccggtgtttattcttatttaacgccttatttatcacacggtcggtatttcaaaccattaaatttaggtcagaagatgaaattaactaaaatatatttgaaaaagttttctcgcgttctttgtcttgcgattggatttgcatcagcatttacatatagttatataacccaacctaagccggaggttaaaaaggtagtctctcagacctatgattttgataaattcactattgactcttctcagcgtcttaatctaagctatcgctatgttttcaaggattctaagggaaaattaattaatagcgacgatttacagaagcaaggttattcactcacatatattgatttatgtactgtttccattaaaaaaggtaattcaaatgaaattgttaaatgtaattaattttgttttcttgatgtttgtttcatcatcttcttttgctcaggtaattgaaatgaataattcgcctctgcgcgattttgtaacttggtattcaaagcaatcaggcgaatccgttattgtttctcccgatgtaaaaggtactgttactgtatattcatctgacgttaaacctgaaaatctacgcaatttctttatttctgttttacgtgcaaataattttgatatggtaggttctaacccttccattattcagaagtataatccaaacaatcaggattatattgatgaattgccatcatctgataatcaggaatatgatgataattccgctccttctggtggtttctttgttccgcaaaatgataatgttactcaaacttttaaaattaataacgttcgggcaaaggatttaatacgagttgtcgaattgtttgtaaagtctaatacttctaaatcctcaaatgtattatctattgacggctctaatctattagttgttagtgctcctaaagatattttagataaccttcctcaattcctttcaactgttgatttgccaactgaccagatattgattgagggtttgatatttgaggttcagcaaggtgatgctttagatttttcatttgctgctggctctcagcgtggcactgttgcaggcggtgttaatactgaccgcctcacctctgttttatcttctgctggtggttcgttcggtatttttaatggcgatgttttagggctatcagttcgcgcattaaagactaatagccattcaaaaatattgtctgtgccacgtattcttacgctttcaggtcagaagggttctatctctgttggccagaatgtcccttttattactggtcgtgtgactggtgaatctgccaatgtaaataatccatttcagacgattgagcgtcaaaatgtaggtatttccatgagcgtttttcctgttgcaatggctggcggtaatattgttctggatattaccagcaaggccgatagtttgagttcttctactcaggcaagtgatgttattactaatcaaagaagtattgctacaacggttaatttgcgtgatggacagactcttttactcggtggcctcactgattataaaaacacttctcaggattctggcgtaccgttcctgtctaaaatccctttaatcggcctcctgtttagctcccgctctgattctaacgaggaaagcacgttatacgtgctcgtcaaagcaaccatagtacgcgccctgtagcggcgcattaagcgcggcgggtgtggtggttacgcgcagcgtgaccgctacacttgccagcgccctagcgcccgctcctttcgctttcttcccttcctttctcgccacgttcgccggctttccccgtcaagctctaaatcgggggctccctttagggttccgatttagtgctttacggcacctcgaccccaaaaaacttgatttgggtgatggttcacgtagtgggccatcgccctgatagacggtttttcgccctttgacgttggagtccacgttctttaatagtggactcttgttccaaactggaacaacactcaaccctatctcgggctattcttttgatttataagggattttgccgatttcggaaccaccatcaaacaggattttcgcctgctggggcaaaccagcgtggaccgcttgctgcaactctctcagggccaggcggtgaagggcaatcagctgttgcccgtctcactggtgaaaagaaaaaccaccctggcgcccaatacgcaaaccgcctctccccgcgcgttggccgattcattaatgcagctggcacgacaggtttcccgactggaaagcgggcagtgagcgcaacgcaattaatgtgagttagctcactcattaggcaccccaggctttacactttatgcttccggctcgtatgttgtgtggaattgtgagcggataacaatttcacacaggaaacagctatgaccatgattacgaattcgagctctgactactgcttggattctcaccaataaaaaacgcccggcggcaaccgagcgttctgaacaaatccagatggagttctgaggtcattactggatctatcaacaggagtccaagccaattctcgaacgtttcaattcagcggcaacgggttgccgtgataacggctggcaaagaacagcagcggctggggggcattcgcctccggcactccacaggcgctaacgcgcgcaatgaagagcgtgtggtcgtgtacttcaaccgtgctctccacctcgcattcgaaccaggccatggcgtcccgcagagtggggaggccggcctgaactgtgaaagcaggaggaggagtgccatcgatcacacgcttgctgaagaatgccgataacatcttctgactttcacccaggaggctgacgccgaagcgtccgccttgagtcagcagctcatgcatacggcccgacttcagggacaccatcacagtcggcgggtccagactgatggaggtgaagctgttcaccgtcatgccatgcacttcgccctcgtcagtctccgcgctgagaaccgcaattcccgtcgcgaacagtgcaaccgcctggcggaagctggtggagtcgatatccaccaccacatctttttttaacgtcatttgaatcacccaggagttagggctccgctggccttgaccagcggagcaatagcgtcaggccgcaatagtgggtgcgtactggctgcaccactgaccgatacgttccgggctggagaagcgatcccactgaagttccggatagttgaagttgtccgtgaactcatcagccatttcacggctctggctcaggatctgaaggaaggtgaggaattccggcggaagttccgtgaaggcgctcagagtgaagttggtccagcgggtggcgcacagcacgcgatcctggcggcgacgctccaggtgttcgctgaagcgcaggtcgtagacagagtgcgcaaggatttcctcgcccagaatccatgccgcataggacgccatgttcgcgccctggcccaagaccggatcgacagttgcctggatgtcgcccagcccgatgatggttttgccgttattgagggtcgcatgaccgtcgcggaatactggcacaacaccgccctggaggatgtccagagaactgttggccaggtcgaactcagccggatcgatgcgctcggcaacggaaggatgatgcttacgcagcttctccagcatcagatcgaggaacgcacgcgggtcatcgtcatacttggtgtgggcgaggacttccagatcgctaccaatatggttttcgagcaccagcgctgtgctcatgccattgaacgacagggttggaatctcaatcagctcgccatgccctggcgagaaggacatagtcaccgcgcgaatcggtgcttccttgatgcccttgaagagaccaacgcacagtgcccgttgcggcttctcgaagggcgagttttcggactgcttctcgaacaccttgccgagggcgtatttaccagtgcacacaaccagcagatcatactgctccgacagcccttccagatcttcggcagacacggcgtcgtagcagaacttgccgcccctggcttccagtgcacgcatcagcatcggcaggtagagacggtagtccactgcacggctgggagccttgagatcaccgtagaaacgcatgggctgcggcccacctacgtagtagtagtggccgaaatagccaaactcctcagacggccactcattgacgtcgagggcaacctcccgctgcaccgtcaccgcgttgtgagcaacggtattcaggagccgcagtccactgtactcatcgggcttacgatcagtgtacacagtgacgtcgacgtcatgctggcggaggaagaggccaagatggaggccggcagtgcctgcaccaacaataccgatacgctttttcatgcatgctacctccttaatccttcagctgggtcagtgcgtcctgctgatgtgctcagtatctctatcactgatagggatgtcaatctctatcactgatagggaggtacccggggatcctctagagtcgacctgcaggcatgcaagcttggcactggccgtcgttttacaacgtcgtgactgggaaaaccctggcgttacccaacttaatcgccttgcagcacatccccctttcgccagctggcgtaatagcgaagaggcccgcaccgatcgcccttcccaacagttgcgcagcctgaatggcgaatggcgctttgcctggtttccggcaccagaagcggtgccggaaagctggctggagtgcgatcttcctgaggccgatactgtcgtcgtcccctcaaactggcagatgcacggttacgatgcgcccatctacaccaacgtgacctatcccattacggtcaatccgccgtttgttcccacggagaatccgacgggttgttactcgctcacatttaatgttgatgaaagctggctacaggaaggccagacgcgaattatttttgatggcgttcctattggttaaaaaatgagctgatttaacaaaaatttaatgcgaattttaacaaaatattaacgtttacaatttaaatatttgcttatacaatcttcctgtttttggggcttttctgattatcaaccggggtacatatgattgacatgctagttttacgattaccgttcatcgattctcttgtttgctccagactctcaggcaatgacctgatagcctttgtagatctctcaaaaatagctaccctctccggcattaatttatcagctagaacggttgaatatcatattgatggtgatttgactgtctccggcctttctcacccttttgaatctttacctacacattactcaggcattgcatttaaaatatatgagggttctaaaaatttttatccttgcgttgaaataaaggcttctcccgcaaaagtattacagggtcataatgtttttggtacaaccgatttagctttatgctctgaggctttattgcttaattttgctaattctttgccttgcctgtatgatttattggatgtt

SEQ ID NO: 7 - DNA, 3101 bp, Artificial Sequence
  Synthetic Polynucleotide
gacgtctgtgcaagtactactgttctgcagtcacttgaattcgatacccagctgggtggagtgcaccaaggagcatgcgaaggaaacgtttcgcagaagcttccgcaaggtaccactttgccgcggagtatttgtacatttgaaggatcctcaagtcggccgcccgttccatggatactcgtcgaccattacgctagccgtctggagctcggactgcttaagtcgctccatatgctgaaatgagctgttgacaattaatcatccggctcgtataatgtgtggaattgtgagcggataacaatttcacaccccgggataaggaggacaattgatgcgtaaaggagaagaacttttcactggagttgtcccaattcttgttgaattagatggtgatgttaatgggcacaaattttctgtcagtggagagggtgaaggtgatgcaacatacggaaaacttacccttaaatttatttgcactactggaaaactacctgttccgtggccaacacttgtcactactttcggttatggtgttcaatgctttgcgagatacccagatcacatgaaacagcatgactttttcaagagtgccatgcccgaaggttacgtacaggaaagaactatatttttcaaagatgacgggaactacaagacacgtgctgaagtcaagtttgaaggtgatacccttgttaatagaatcgagttaaaaggtattgattttaaagaagatggaaacattcttggacacaaattggaatacaactataactcacacaatgtatacatcatggcagacaaacaaaagaatggaatcaaagttaacttcaaaattagacacaacattgaagatggaagcgttcaactagcagaccattatcaacaaaatactccgattggcgatggccctgtccttttaccagacaaccattacctgtccacacaatctgccctttcgaaagatcccaacgaaaagagagaccacatggtccttcttgagtttgtaaccgctgctgggattacacatggcatggatgaactatacaaataaggcgccagggttgatatctatcgccctagggaccgtctcgagagaatcaatattaatccaacgcgtggcatcaaataaaacgaaaggctcagtcgaaagactgggcctttcgttttatctgttgtttgtcggtgaacgctctcctgagtaggacaaatccgccgccctagacttaggcgttcggctgcggcgagcggtatcagctcactcaaaggcggtaatacggttatccacagaatcaggggataacgcaggaaagaacatgtgagcaaaaggccagcaaaaggccaggaaccgtaaaaaggccgcgttgctggcgtttttccataggctccgcccccctgacgagcatcacaaaaatcgacgctcaagtcagaggtggcgaaacccgacaggactataaagataccaggcgtttccccctggaagctccctcgtgcgctctcctgttccgaccctgccgcttaccggatacctgtccgcctttctcccttcgggaagcgtggcgctttctcatagctcacgctgtaggtatctcagttcggtgtaggtcgttcgctccaagctgggctgtctgcacgaaccccccgttcagcccgaccgctgcgccttatccggtaactatcgtcttgagtccaacccggtaagacacgacttatcgccactggcagcagccactggtaacaggattagcagagcgaggtatgtaggcggtgctacagagttcttgaagtggtggcctaactacggctacactagaaggacagtatttggtatctgcgctctgctgaagccagttaccttcggaaaaagagttggtagctcttgatccggcaaacaaaccaccgctggtagcggtggtttttttgtttgcaagcagcagattacgcgcagaaaaaaaggatctcaagaagatcctttgatcttttctacggggtctgacgctcagtggaacgaaaactcacgttaagggattttggtcatggctagtgcttggattctcaccaataaaaaacgcccggcggcaaccgagcgttctgaacaaatccagatggagttctgaggtcattactggatctatcaacaggagtccaagccaattctcgaaccccagagtcccgctcagaagaactcgtcaagaaggcgatagaaggcgatgcgctgcgaatcgggagcggcgataccgtaaagcacgaggaagcggtcagcccattcgccgccaagctcttcagcaatatcacgggtagccaacgctatgtcctgatagcggtccgccacacccagccggccacagtcgatgaatccagaaaagcggccattttccaccatgatattcggcaagcaggcatcgccgtgggtcacgacgagatcctcgccgtcgggcatacgcgccttgagcctggcgaacagttcggctggcgcgagcccctgatgctcttcgtccagatcatcctgatcgacaagaccggcttccatccgagtacgtgctcgctcgatgcgatgtttcgcttggtggtcgaatgggcaggtagccggatcaagcgtatgcagccgccgcattgcatcagccatgatggatactttctcggcaggagcaaggtgagatgacaggagatcctgccccggcacttcgcccaatagcagccagtcccttcccgcttcagtgacaacgtcgagcacagccgcgcaaggaacgcccgtcgtggccagccacgatagccgcgctgcctcgtcttgcagttcattcagggcaccggacaggtcggtcttgacaaaaagaaccgggcgaccctgcgctgacagccggaacacggcggcatcagagcagccgattgtctgttgtgcccagtcatagccgaatagcctctccacccaagccgccggagaacctgcgtgcaatccatcttgttcaatcatgcgaaacgatcctcatcctgtctcttgatcagatcttgatcccctgcgccatcagatccttggcggcaagaaagccatccagtttactttgcagggcttcccaaccttaccagagggcggcccaactggcaattcc

SEQ ID NO: 8 - DNA, 3524 bp, Artificial Sequence
  Synthetic Polynucleotide
gacgtctgtgcaagtactactgttctgcagtcacttgaattcgatacccagctgggtggagtgcaccaaggagcatgcgaaggaaacgtttcgcagaagcttccgcaaggtaccactttgccgcggagtatttgtacatttgaaggatcctcaagtcggccgcccgttccatggatactcgtcgaccattacgctagccgtctggagctcggactgcttaagtcgctccatatgctgaaatgagctgttgacaattaatcatccggctcgtataatgtgtggaattgtgagcggataacaatttcacaccccgggataaggaggacaattgatgcgtaaaggagaagaacttttcactggagttgtcccaattcttgttgaattagatggtgatgttaatgggcacaaattttctgtcagtggagagggtgaaggtgatgcaacatacggaaaacttacccttaaatttatttgcactactggaaaactacctgttccgtggccaacacttgtcactactttcggttatggtgttcaatgctttgcgagatacccagatcacatgaaacagcatgactttttcaagagtgccatgcccgaaggttacgtacaggaaagaactatatttttcaaagatgacgggaactacaagacacgtgctgaagtcaagtttgaaggtgatacccttgttaatagaatcgagttaaaaggtattgattttaaagaagatggaaacattcttggacacaaattggaatacaactataactcacacaatgtatacatcatggcagacaaacaaaagaatggaatcaaagttaacttcaaaattagacacaacattgaagatggaagcgttcaactagcagaccattatcaacaaaatactccgattggcgatggccctgtccttttaccagacaaccattacctgtccacacaatctgccctttcgaaagatcccaacgaaaagagagaccacatggtccttcttgagtttgtaaccgctgctgggattacacatggcatggatgaactatacaaataaggcgccagggttgatatctatcgccctagggaccgtctcgagagcgccctgtagcggcgcattaagcgcggcgggtgtggtggttacgcgcagcgtgaccgctacacttgccagcgccctagcgcccgctcctttcgctttcttcccttcctttctcgccacgttcgccggctttccccgtcaagctctaaatcgggggctccctttagggttccgatttagtgctttacggcacctcgaccccaaaaaacttgattagggtgatggttcacgtagtgggccatcgccctgatagacggtttttcgccctttgacgttggagtccacgttctttaatagtggactcttgttccaaactggaacaacactcaaccctatctcggtctattcttttgatttataagggattttgccgatttcggcctattggttaaaaaatgagctgatttaacaaaaatttaacgcgaattaaatattaatccaacgcgtggcatcaaataaaacgaaaggctcagtcgaaagactgggcctttcgttttatctgttgtttgtcggtgaacgctctcctgagtaggacaaatccgccgccctagacttaggcgttcggctgcggcgagcggtatcagctcactcaaaggcggtaatacggttatccacagaatcaggggataacgcaggaaagaacatgtgagcaaaaggccagcaaaaggccaggaaccgtaaaaaggccgcgttgctggcgtttttccataggctccgcccccctgacgagcatcacaaaaatcgacgctcaagtcagaggtggcgaaacccgacaggactataaagataccaggcgtttccccctggaagctccctcgtgcgctctcctgttccgaccctgccgcttaccggatacctgtccgcctttctcccttcgggaagcgtggcgctttctcatagctcacgctgtaggtatctcagttcggtgtaggtcgttcgctccaagctgggctgtctgcacgaaccccccgttcagcccgaccgctgcgccttatccggtaactatcgtcttgagtccaacccggtaagacacgacttatcgccactggcagcagccactggtaacaggattagcagagcgaggtatgtaggcggtgctacagagttcttgaagtggtggcctaactacggctacactagaaggacagtatttggtatctgcgctctgctgaagccagttaccttcggaaaaagagttggtagctcttgatccggcaaacaaaccaccgctggtagcggtggtttttttgtttgcaagcagcagattacgcgcagaaaaaaaggatctcaagaagatcctttgatcttttctacggggtctgacgctcagtggaacgaaaactcacgttaagggattttggtcatggctagtgcttggattctcaccaataaaaaacgcccggcggcaaccgagcgttctgaacaaatccagatggagttctgaggtcattactggatctatcaacaggagtccaagccaattctcgaaccccagagtcccgctcagaagaactcgtcaagaaggcgatagaaggcgatgcgctgcgaatcgggagcggcgataccgtaaagcacgaggaagcggtcagcccattcgccgccaagctcttcagcaatatcacgggtagccaacgctatgtcctgatagcggtccgccacacccagccggccacagtcgatgaatccagaaaagcggccattttccaccatgatattcggcaagcaggcatcgccgtgggtcacgacgagatcctcgccgtcgggcatacgcgccttgagcctggcgaacagttcggctggcgcgagcccctgatgctcttcgtccagatcatcctgatcgacaagaccggcttccatccgagtacgtgctcgctcgatgcgatgtttcgcttggtggtcgaatgggcaggtagccggatcaagcgtatgcagccgccgcattgcatcagccatgatggatactttctcggcaggagcaaggtgagatgacaggagatcctgccccggcacttcgcccaatagcagccagtcccttcccgcttcagtgacaacgtcgagcacagccgcgcaaggaacgcccgtcgtggccagccacgatagccgcgctgcctcgtcttgcagttcattcagggcaccggacaggtcggtcttgacaaaaagaaccgggcgaccctgcgctgacagccggaacacggcggcatcagagcagccgattgtctgttgtgcccagtcatagccgaatagcctctccacccaagccgccggagaacctgcgtgcaatccatcttgttcaatcatgcgaaacgatcctcatcctgtctcttgatcagatcttgatcccctgcgccatcagatccttggcggcaagaaagccatccagtttactttgcagggcttcccaaccttaccagagggcggcccaactggcaattcc

SEQ ID NO: 9 - DNA, 7413 bp, Artificial Sequence
  Synthetic Polynucleotide
aatgctactactattagtagaattgatgccaccttttcagctcgcgccccaaatgaaaatatagctaaacaggttattgaccatttgcgaaatgtatctaatggtcaaactaaatctactcgttcgcagaattgggaatcaactgttatatggaatgaaacttccagacaccgtactttagttgcatatttaaaacatgttgagctacagcattatattcagcaattaagctctaagccatccgcaaaaatgacctcttatcaaaaggagcaattaaaggtactctctaatcctgacctgttggagtttgcttccggtctggttcgctttgaagctcgaattaaaacgcgatatttgaagtctttcgggcttcctcttaatctttttgatgcaatccgctttgcttctgactataatagtcagggtaaagacctgatttttgatttatggtcattctcgttttctgaactgtttaaagcatttgagggggattcaatgaatatttatgacgattccgcagtattggacgctatccagtctaaacattttactattaccccctctggcaaaacttcttttgcaaaagcctctcgctattttggtttttatcgtcgtctggtaaacgagggttatgatagtgttgctcttactatgcctcgtaattccttttggcgttatgtatctgcattagttgaatgtggtattcctaaatctcaactgatgaatctttctacctgtaataatgttgttccgttagttcgttttattaacgtagatttttcttcccaacgtcctgactggtataatgagccagttcttaaaatcgcataaggtaattcacaatgattaaagttgaaattaaaccatctcaagcccaatttactactcgttctggtgtttctcgtcagggcaagccttattcactgaatgagcagctttgttacgttgatttgggtaatgaatatccggttcttgtcaagattactcttgatgaaggtcagccagcctatgcgcctggtctgtacaccgttcatctgtcctctttcaaagttggtcagttcggttcccttatgattgaccgtctgcgcctcgttccggctaagtaacatggagcaggtcgcggatttcgacacaatttatcaggcgatgatacaaatctccgttgtactttgtttcgcgcttggtataatcgctgggggtcaaagatgagtgttttagtgtattcttttgcctctttcgttttaggttggtgccttcgtagtggcattacgtattttacccgtttaatggaaacttcctcatgaaaaagtctttagtcctcaaagcctctgtagccgttgctaccctcgttccgatgctgtctttcgctgctgagggtgacgatcccgcaaaagcggcctttaactccctgcaagcctcagcgaccgaatatatcggttatgcgtgggcgatggttgttgtcattgtcggcgcaactatcggtatcaagctgtttaagaaattcacctcgaaagcaagctgataaaccgatacaattaaaggctccttttggagccttttttttggagattttcaacgtgaaaaaattattattcgcaattcctttagttgttcctttctattctcactccgctgaaactgttgaaagttgtttagcaaaatcccatacagaaaattcatttactaacgtctggaaagacgacaaaactttagatcgttacgctaactatgagggctgtctgtggaatgctacaggcgttgtagtttgtactggtgacgaaactcagtgttacggtacatgggttcctattgggcttgctatccctgaaaatgagggtggtggctctgagggtggcggttctgagggtggcggttctgagggtggcggtactaaacctcctgagtacggtgatacacctattccgggctatacttatatcaaccctctcgacggcacttatccgcctggtactgagcaaaaccccgctaatcctaatccttctcttgaggagtctcagcctcttaatactttcatgtttcagaataataggttccgaaataggcagggggcattaactgtttatacgggcactgttactcaaggcactgaccccgttaaaacttattaccagtacactcctgtatcatcaaaagccatgtatgacgcttactggaacggtaaattcagagactgcgctttccattctggctttaatgaggatttatttgtttgtgaatatcaaggccaatcgtctgacctgcctcaacctcctgtcaatgctggcggcggctctggtggtggttctggtggcggctctgagggtggtggctctgagggtggcggttctgagggtggcggctctgagggaggcggttccggtggtggctctggttccggtgattttgattatgaaaagatggcaaacgctaataagggggctatgaccgaaaatgccgatgaaaacgcgctacagtctgacgctaaaggcaaacttgattctgtcgctactgattacggtgctgctatcgatggtttcattggtgacgtttccggccttgctaatggtaatggtgctactggtgattttgctggctctaattcccaaatggctcaagtcggtgacggtgataattcacctttaatgaataatttccgtcaatatttaccttccctccctcaatcggttgaatgtcgcccttttgtctttggcgctggtaaaccatatgaattttctattgattgtgacaaaataaacttattccgtggtgtctttgcgtttcttttatatgttgccacctttatgtatgtattttctacgtttgctaacatactgcgtaataaggagtcttaatcatgccagttcttttgggtattccgttattattgcgtttcctcggtttccttctggtaactttgttcggctatctgcttacttttcttaaaaagggcttcggtaagatagctattgctatttcattgtttcttgctcttattattgggcttaactcaattcttgtgggttatctctctgatattagcgctcaattaccctctgactttgttcagggtgttcagttaattctcccgtctaatgcgcttccctgtttttatgttattctctctgtaaaggctgctattttcatttttgacgttaaacaaaaaatcgtttcttatttggattgggataaataatatggctgtttattttgtaactggcaaattaggctctggaaagacgctcgttagcgttggtaagattcaggataaaattgtagctgggtgcaaaatagcaactaatcttgatttaaggcttcaaaacctcccgcaagtcgggaggttcgctaaaacgcctcgcgttcttagaataccggataagccttctatatctgatttgcttgctattgggcgcggtaatgattcctacgatgaaaataaaaacggcttgcttgttctcgatgagtgcggtacttggtttaatacccgttcttggaatgataaggaaagacagccgattattgattggtttctacatgctcgtaaattaggatgggatattatttttcttgttcaggacttatctattgttgataaacaggcgcgttctgcattagctgaacatgttgtttattgtcgtcgtctggacagaattactttaccttttgtcggtactttatattctcttattactggctcgaaaatgcctctgcctaaattacatgttggcgttgttaaatatggcgattctcaattaagccctactgttgagcgttggctttatactggtaagaatttgtataacgcatatgatactaaacaggctttttctagtaattatgattccggtgtttattcttatttaacgccttatttatcacacggtcggtatttcaaaccattaaatttaggtcagaagatgaaattaactaaaatatatttgaaaaagttttctcgcgttctttgtcttgcgattggatttgcatcagcatttacatatagttatataacccaacctaagccggaggttaaaaaggtagtctctcagacctatgattttgataaattcactattgactcttctcagcgtcttaatctaagctatcgctatgttttcaaggattctaagggaaaattaattaatagcgacgatttacagaagcaaggttattcactcacatatattgatttatgtactgtttccattaaaaaaggtaattcaaatgaaattgttaaatgtaattaattttgttttcttgatgtttgtttcatcatcttcttttgctcaggtaattgaaatgaataattcgcctctgcgcgattttgtaacttggtattcaaagcaatcaggcgaatccgttattgtttctcccgatgtaaaaggtactgttactgtatattcatctgacgttaaacctgaaaatctacgcaatttctttatttctgttttacgtgcaaataattttgatatggtaggttctaacccttccattattcagaagtataatccaaacaatcaggattatattgatgaattgccatcatctgataatcaggaatatgatgataattccgctccttctggtggtttctttgttccgcaaaatgataatgttactcaaacttttaaaattaataacgttcgggcaaaggatttaatacgagttgtcgaattgtttgtaaagtctaatacttctaaatcctcaaatgtattatctattgacggctctaatctattagttgttagtgctcctaaagatattttagataaccttcctcaattcctttcaactgttgatttgccaactgaccagatattgattgagggtttgatatttgaggttcagcaaggtgatgctttagatttttcatttgctgctggctctcagcgtggcactgttgcaggcggtgttaatactgaccgcctcacctctgttttatcttctgctggtggttcgttcggtatttttaatggcgatgttttagggctatcagttcgcgcattaaagactaatagccattcaaaaatattgtctgtgccacgtattcttacgctttcaggtcagaagggttctatctctgttggccagaatgtcccttttattactggtcgtgtgactggtgaatctgccaatgtaaataatccatttcagacgattgagcgtcaaaatgtaggtatttccatgagcgtttttcctgttgcaatggctggcggtaatattgttctggatattaccagcaaggccgatagtttgagttcttctactcaggcaagtgatgttattactaatcaaagaagtattgctacaacggttaatttgcgtgatggacagactcttttactcggtggcctcactgattataaaaacacttctcaggattctggcgtaccgttcctgtctaaaatccctttaatcggcctcctgtttagctcccgctctgattctaacgaggaaagcacgttatacgtgctcgtcaaagcaaccatagtacgcgccctgtagcggcgcattaagcgcggcgggtgtggtggttacgcgcagcgtgaccgctacacttgccagcgccctagcgcccgctcctttcgctttcttcccttcctttctcgccacgttcgccggctttccccgtcaagctctaaatcgggggctccctttagggttccgatttagtgctttacggcacctcgaccccaaaaaacttgatttgggtgatggttcacgtagtgggccatcgccctgatagacggtttttcgccctttgacgttggagtccacgttctttaatagtggactcttgttccaaactggaacaacactcaaccctatctcgggctattcttttgatttataagggattttgccgatttcgggactgcttaagtcgctccatatgctgaaatgagctgttgacaattaatcatccggctcgtataatgtgtggaattgtgagcggataacaatttcacaccccgggataaggaggacaattgatgcgtaaaggagaagaacttttcactggagttgtcccaattcttgttgaattagatggtgatgttaatgggcacaaattttctgtcagtggagagggtgaaggtgatgcaacatacggaaaacttacccttaaatttatttgcactactggaaaactacctgttccgtggccaacacttgtcactactttcggttatggtgttcaatgctttgcgagatacccagatcacatgaaacagcatgactttttcaagagtgccatgcccgaaggttacgtacaggaaagaactatatttttcaaagatgacgggaactacaagacacgtgctgaagtcaagtttgaaggtgatacccttgttaatagaatcgagttaaaaggtattgattttaaagaagatggaaacattcttggacacaaattggaatacaactataactcacacaatgtatacatcatggcagacaaacaaaagaatggaatcaaagttaacttcaaaattagacacaacattgaagatggaagcgttcaactagcagaccattatcaacaaaatactccgattggcgatggccctgtccttttaccagacaaccattacctgtccacacaatctgccctttcgaaagatcccaacgaaaagagagaccacatggtccttcttgagtttgtaaccgctgctgggattacacatggcatggatgaactatacaaataaggcgccagggttgatatctatcgccctagggaccgtctcgagagaatcaatattaatccaacgcgtggcatcaaataaaacgaaaggctcagtcgaaagactgggcctttcgttttatctgttgtttgtcggtgaacgctctcctgagtaggacaaatccgccgccctagactattggttaaaaaatgagctgatttaacaaaaatttaatgcgaattttaacaaaatattaacgtttacaatttaaatatttgcttatacaatcttcctgtttttggggcttttctgattatcaaccggggtacatatgattgacatgctagttttacgattaccgttcatcgattctcttgtttgctccagactctcaggcaatgacctgatagcctttgtagatctctcaaaaatagctaccctctccggcattaatttatcagctagaacggttgaatatcatattgatggtgatttgactgtctccggcctttctcacccttttgaatctttacctacacattactcaggcattgcatttaaaatatatgagggttctaaaaatttttatccttgcgttgaaataaaggcttctcccgcaaaagtattacagggtcataatgtttttggtacaaccgatttagctttatgctctgaggctttattgcttaattttgctaattctttgccttgcctgtatgatttattggatgtt